European Patent Specification EP 4 066 869 B1, published July 2, 2025. Title: METHOD FOR FIBROCARTILAGE RECONSTRUCTION USING MECHANICAL STIMULATION. Applicant: University-Industry Cooperation Group of Kyung Hee University. The sequence listing filed with the application follows.

SEQUENCE LISTING (4 sequences)

SEQ ID NO: 1 - DNA, 20 bp, Artificial Sequence
  Sox-9 forward
ctccgacaccgagaatacac

SEQ ID NO: 2 - DNA, 20 bp, Artificial Sequence
  Sox-9 reverse
ccattcttcaccgacttcct

SEQ ID NO: 3 - DNA, 20 bp, Artificial Sequence
  GAPDH forward
tcaccatcttccaggagcga

SEQ ID NO: 4 - DNA, 20 bp, Artificial Sequence
  GAPDH reverse
cacaatgccgaagtggtcgt